European Patent Application EP 4 717 273 A2, published April 1, 2026. Title: ANTI-LY6G6D ANTIBODIES AND METHODS OF USE. Applicant: Genentech Inc. The sequence listing filed with the application follows.

SEQUENCE LISTING (147 sequences)

SEQ ID NO: 1 - protein, 11 aa, synthetic construct
  REGION 1..11: note = Synthetic Construct
QASESITRYLN

SEQ ID NO: 2 - protein, 7 aa, synthetic construct
  REGION 1..7: note = Synthetic Construct
DASKLPS

SEQ ID NO: 3 - protein, 13 aa, synthetic construct
  REGION 1..13: note = Synthetic Construct
QSTSFRGRSYQNT

SEQ ID NO: 4 - protein, 5 aa, synthetic construct
  REGION 1..5: note = Synthetic Construct
NNAMI

SEQ ID NO: 5 - protein, 17 aa, synthetic construct
  REGION 1..17: note = Synthetic Construct
ALSFADNTAYYATWASG

SEQ ID NO: 6 - skipped

SEQ ID NO: 7 - protein, 442 aa, synthetic construct
  REGION 1..442: note = Synthetic Construct
EVQLLESGGGLVQPGGSLRLSCAASGFDFVNNAMIWVREAPGKGLEWVSALSFADNTAYYATWASGRFTISRDSSKTTVYLQMNSLRAEDTAVYYCMRGDLWGPGTLVTVSSASTKGPSVFPLAPSSKSTSGGTAALGCLVKDYFPEPVTVSWNSGALTSGVHTFPAVLQSSGLYSLKSVVTVPSSSLGTQTYICNVNHKPSNTKVDKKVEPKSCDKTHTCPPCPAPELLGGPSVFLFPPKPKDTLMISRTPEVTCVVVDVSHEDPEVKFNWYVDGVEVHNAKTKPREEQYGSTYRVVSVLTVLHQDWLNGKEYKCKVSNKALPAPIEKTISKAKGQPREPQVYTLPPSREEMTKNQVSLWCLVKGFYPSDIAVEWESNGQPENNYKTTPPVLDSDGSFFLYSKLTVDKSRWQQGNVFSCSVMHEALHNHYTQKSLSLSPGK

SEQ ID NO: 8 - protein, 442 aa, synthetic construct
  REGION 1..442: note = Synthetic Construct
EVQLLESGGGLVQPGGSLRLSCAASGFDFVNNAMIWVREAPGKGLEWVSALSFADNTAYYATWASGRFTISRDSSKTTVYLQMNSLRAEDTAVYYCMRGDLWGPGTLVTVSSASTKGPSVFPLAPSSKSTSGGTAALGCLVKDYFPEPVTVSWNSGALTSGVHTFPAVLQSSGLYSLKSVVTVPSSSLGTQTYICNVNHKPSNTKVDKKVEPKSCDKTHTCPPCPAPELLGGPSVFLFPPKPKDTLMISRTPEVTCVVVDVSHEDPEVKFNWYVDGVEVHNAKTKPREEQYGSTYRVVSVLTVLHQDWLNGKEYKCKVSNKALPAPIEKTISKAKGQPREPQVYTLPPSREEMTKNQVSLSCAVKGFYPSDIAVEWESNGQPENNYKTTPPVLDSDGSFFLVSKLTVDKSRWQQGNVFSCSVMHEALHNHYTQKSLSLSPGK

SEQ ID NO: 9 - protein, 218 aa, synthetic construct
  REGION 1..218: note = Synthetic Construct
DIQMTQSPSTLSASVGDRVTITCQASESITRYLNWYQKKPGKAPKLLIYDASKLPSGVPSRFSGSGSGTEFTLTISSLQPDDFATYYCQSTSFRGRSYQNTFGGGTKVEIKRTVAAPSVFIFPPSDEQLKSGTASVECLLNNFYPREAKVQWKVDNALQSGNSQESVTEQDSKDSTYSLSSTLTLSKADYEKHKVYACEVTHQGLSSPVTKSFNRGEC

SEQ ID NO: 10 - protein, 112 aa, synthetic construct
  REGION 1..112: note = Synthetic Construct
EVQLLESGGGLVQPGGSLRLSCAASGFDFVNNAMIWVREAPGKGLEWVSALSFADNTAYYATWASGRFTISRDSSKTTVYLQMNSLRAEDTAVYYCMRGDLWGPGTLVTVSS

SEQ ID NO: 11 - protein, 111 aa, synthetic construct
  REGION 1..111: note = Synthetic Construct
DIQMTQSPSTLSASVGDRVTITCQASESITRYLNWYQKKPGKAPKLLIYDASKLPSGVPSRFSGSGSGTEFTLTISSLQPDDFATYYCQSTSFRGRSYQNTFGGGTKVEIK

SEQ ID NO: 12 - protein, 17 aa, synthetic construct
  REGION 1..17: note = Synthetic Construct
KSSQSLLNSRTRKNYLA

SEQ ID NO: 13 - protein, 7 aa, synthetic construct
  REGION 1..7: note = Synthetic Construct
WASTRES

SEQ ID NO: 14 - protein, 8 aa, synthetic construct
  REGION 1..8: note = Synthetic Construct
TQSFILRT

SEQ ID NO: 15 - protein, 5 aa, synthetic construct
  REGION 1..5: note = Synthetic Construct
SYYIH

SEQ ID NO: 16 - protein, 17 aa, synthetic construct
  REGION 1..17: note = Synthetic Construct
WIYPENDNTKYNEKFKD

SEQ ID NO: 17 - protein, 10 aa, synthetic construct
  REGION 1..10: note = Synthetic Construct
DGYSRYYFDY

SEQ ID NO: 18 - protein, 449 aa, synthetic construct
  REGION 1..449: note = Synthetic Construct
EVQLVQSGAEVKKPGASVKVSCKASGFTFTSYYIHWVRKAPGQGLEWIGWIYPENDNTKYNEKFKDRVTITADTSTSTAYLELSSLRSEDTAVYYCARDGYSRYYFDYWGQGTLVTVSSASTKGPSVFPLAPSSKSTSGGTAALGCLVKDYFPEPVTVSWNSGALTSGVHTFPAVLQSSGLYSLESVVTVPSSSLGTQTYICNVNHKPSNTKVDKKVEPKSCDKTHTCPPCPAPELLGGPSVFLFPPKPKDTLMISRTPEVTCVVVDVSHEDPEVKFNWYVDGVEVHNAKTKPREEQYGSTYRVVSVLTVLHQDWLNGKEYKCKVSNKALPAPIEKTISKAKGQPREPQVYTLPPSREEMTKNQVSLSCAVKGFYPSDIAVEWESNGQPENNYKTTPPVLDSDGSFFLVSKLTVDKSRWQQGNVFSCSVMHEALHNHYTQKSLSLSPGK

SEQ ID NO: 19 - protein, 219 aa, synthetic construct
  REGION 1..219: note = Synthetic Construct
DIVMTQSPDSLAVSLGERATINCKSSQSLLNSRTRKNYLAWYQEKPGQPPKLLIYWASTRESGVPDRFSGSGSGTDFTLTISSLQAEDVAVYYCTQSFILRTFGQGTKVEIKRTVAAPSVFIFPPSDEQLKSGTASVKCLLNNFYPREAKVQWKVDNALQSGNSQESVTEQDSKDSTYSLSSTLTLSKADYEKHKVYACEVTHQGLSSPVTKSFNRGEC

SEQ ID NO: 20 - protein, 119 aa, synthetic construct
  REGION 1..119: note = Synthetic Construct
EVQLVQSGAEVKKPGASVKVSCKASGFTFTSYYIHWVRKAPGQGLEWIGWIYPENDNTKYNEKFKDRVTITADTSTSTAYLELSSLRSEDTAVYYCARDGYSRYYFDYWGQGTLVTVSS

SEQ ID NO: 21 - protein, 112 aa, synthetic construct
  REGION 1..112: note = Synthetic Construct
DIVMTQSPDSLAVSLGERATINCKSSQSLLNSRTRKNYLAWYQEKPGQPPKLLIYWASTRESGVPDRFSGSGSGTDFTLTISSLQAEDVAVYYCTQSFILRTFGQGTKVEIK

SEQ ID NO: 22 - protein, 112 aa, synthetic construct
  REGION 1..112: note = Synthetic Construct
EVQLLESGGGLVQPGGSLRLSCAASGFDFVNNAMIWVRQAPGKGLEWVSALSFADNTAYYATWASGRFTISRDSSKTTVYLQMNSLRAEDTAVYYCMRGDLWGPGTLVTVSS

SEQ ID NO: 23 - protein, 111 aa, synthetic construct
  REGION 1..111: note = Synthetic Construct
DIQMTQSPSTLSASVGDRVTITCQASESITRYLNWYQQKPGKAPKLLIYDASKLPSGVPSRFSGSGSGTEFTLTISSLQPDDFATYYCQSTSFRGRSYQNTFGGGTKVEIK

SEQ ID NO: 24 - protein, 16 aa, synthetic construct
  REGION 1..16: note = Synthetic Construct
KSSQSLLDSDGRTYLH

SEQ ID NO: 25 - protein, 7 aa, synthetic construct
  REGION 1..7: note = Synthetic Construct
LVSNLDS

SEQ ID NO: 26 - protein, 9 aa, synthetic construct
  REGION 1..9: note = Synthetic Construct
WQGTHLPFT

SEQ ID NO: 27 - protein, 5 aa, synthetic construct
  REGION 1..5: note = Synthetic Construct
SYWIQ

SEQ ID NO: 28 - protein, 18 aa, synthetic construct
  REGION 1..18: note = Synthetic Construct
EILPGSDNTNYNEKFKGK

SEQ ID NO: 29 - protein, 4 aa, synthetic construct
  REGION 1..4: note = Synthetic Construct
WFAY

SEQ ID NO: 30 - protein, 443 aa, synthetic construct
  REGION 1..443: note = Synthetic Construct
QVQLQQSGAELMKPGASVKISCKASGYTFSSYWIQWIKQRPGHGLEWIGEILPGSDNTNYNEKFKGKATFTADTSSSTAYMQLSSLTSEDSAIYYCAKWFAYWGQGTTVTVSAASTKGPSVFPLAPSSKSTSGGTAALGCLVKDYFPEPVTVSWNSGALTSGVHTFPAVLQSSGLYSLSSVVTVPSSSLGTQTYICNVNHKPSNTKVDKKVEPKSCDKTHTCPPCPAPELLGGPSVFLFPPKPKDTLMISRTPEVTCVVVDVSHEDPEVKFNWYVDGVEVHNAKTKPREEQYGSTYRVVSVLTVLHQDWLNGKEYKCKVSNKALPAPIEKTISKAKGQPREPQVYTLPPSREEMTKNQVSLTCLVKGFYPSDIAVEWESNGQPENNYKTTPPVLDSDGSFFLYSKLTVDKSRWQQGNVFSCSVMHEALHNHYTQKSLSLSPGK

SEQ ID NO: 31 - protein, 219 aa, synthetic construct
  REGION 1..219: note = Synthetic Construct
DIVMTQTPLTLSVTIGHPASISCKSSQSLLDSDGRTYLHWLFQRPGQSPRRLIYLVSNLDSGVPDRFTGSGSGTDFTLKISRVEAEDLGVYYCWQGTHLPFTFGSGTKVEIKRTVAAPSVFIFPPSDEQLKSGTASVVCLLNNFYPREAKVQWKVDNALQSGNSQESVTEQDSKDSTYSLSSTLTLSKADYEKHKVYACEVTHQGLSSPVTKSFNRGEC

SEQ ID NO: 32 - protein, 113 aa, synthetic construct
  REGION 1..113: note = Synthetic Construct
QVQLQQSGAELMKPGASVKISCKASGYTFSSYWIQWIKQRPGHGLEWIGEILPGSDNTNYNEKFKGKATFTADTSSSTAYMQLSSLTSEDSAIYYCAKWFAYWGQGTTVTVSA

SEQ ID NO: 33 - protein, 112 aa, synthetic construct
  REGION 1..112: note = Synthetic Construct
DIVMTQTPLTLSVTIGHPASISCKSSQSLLDSDGRTYLHWLFQRPGQSPRRLIYLVSNLDSGVPDRFTGSGSGTDFTLKISRVEAEDLGVYYCWQGTHLPFTFGSGTKVEIK

SEQ ID NO: 34 - protein, 30 aa, synthetic construct
  REGION 1..30: note = Synthetic Construct
EVQLLESGGGLVQPGGSLRLSCAASGFDFV

SEQ ID NO: 35 - protein, 14 aa, synthetic construct
  REGION 1..14: note = Synthetic Construct
WVREAPGKGLEWVS

SEQ ID NO: 36 - protein, 32 aa, synthetic construct
  REGION 1..32: note = Synthetic Construct
RFTISRDSSKTTVYLQMNSLRAEDTAVYYCMR

SEQ ID NO: 37 - protein, 11 aa, synthetic construct
  REGION 1..11: note = Synthetic Construct
WGPGTLVTVSS

SEQ ID NO: 38 - protein, 23 aa, synthetic construct
  REGION 1..23: note = Synthetic Construct
DIQMTQSPSTLSASVGDRVTITC

SEQ ID NO: 39 - protein, 15 aa, synthetic construct
  REGION 1..15: note = Synthetic Construct
WYQKKPGKAPKLLIY

SEQ ID NO: 40 - protein, 32 aa, synthetic construct
  REGION 1..32: note = Synthetic Construct
GVPSRFSGSGSGTEFTLTISSLQPDDFATYYC

SEQ ID NO: 41 - protein, 10 aa, synthetic construct
  REGION 1..10: note = Synthetic Construct
FGGGTKVEIK

SEQ ID NO: 42 - protein, 30 aa, synthetic construct
  REGION 1..30: note = Synthetic Construct
EVQLVQSGAEVKKPGASVKVSCKASGFTFT

SEQ ID NO: 43 - protein, 14 aa, synthetic construct
  REGION 1..14: note = Synthetic Construct
WVREAPGQGLEWIG

SEQ ID NO: 44 - protein, 32 aa, synthetic construct
  REGION 1..32: note = Synthetic Construct
RVTITADTSTSTAYLELSSLRSEDTAVYYCAR

SEQ ID NO: 45 - protein, 11 aa, synthetic construct
  REGION 1..11: note = Synthetic Construct
WGQGTLVTVSS

SEQ ID NO: 46 - protein, 23 aa, synthetic construct
  REGION 1..23: note = Synthetic Construct
DIVMTQSPDSLAVSLGERATINC

SEQ ID NO: 47 - protein, 15 aa, synthetic construct
  REGION 1..15: note = Synthetic Construct
WYQQKPGQPPKLLIY

SEQ ID NO: 48 - protein, 32 aa, synthetic construct
  REGION 1..32: note = Synthetic Construct
GVPDRFSGSGSGTDFTLTISSLQAEDVAVYYC

SEQ ID NO: 49 - protein, 10 aa, synthetic construct
  REGION 1..10: note = Synthetic Construct
FGQGTKVEIK

SEQ ID NO: 50 - protein, 7 aa, synthetic construct
  REGION 1..7: note = Synthetic Construct
WASTRKS

SEQ ID NO: 51 - protein, 9 aa, synthetic construct
  REGION 1..9: note = Synthetic Construct
KQSFILRTF

SEQ ID NO: 52 - protein, 119 aa, synthetic construct
  REGION 1..119: note = Synthetic Construct
EVQLVQSGAEVKKPGASVKVSCKASGFTFTSYYIHWVRQAPGQGLEWIGWIYPENDNTKYNEKFKDRVTITADTSTSTAYLELSSLRSEDTAVYYCARDGYSRYYFDYWGQGTLVTVSS

SEQ ID NO: 53 - protein, 112 aa, synthetic construct
  REGION 1..112: note = Synthetic Construct
DIVMTQSPDSLAVSLGERATINCKSSQSLLNSRTRKNYLAWYQQKPGQPPKLLIYWASTRESGVPDRFSGSGSGTDFTLTISSLQAEDVAVYYCTQSFILRTFGQGTKVEIK

SEQ ID NO: 54 - skipped

SEQ ID NO: 55 - protein, 112 aa, synthetic construct
  REGION 1..112: note = Synthetic Construct
DIVMTQSPDSLAVSLGERATINCKSSQSLLNSRTRKNYLAWYQEKPGQPPKLLIYWASTRKSGVPDRFSGSGSGTDFTLTISSLQAEDVAVYYCKQSFILRTFGQGTKVEIK

SEQ ID NO: 56 - skipped

SEQ ID NO: 57 - protein, 219 aa, synthetic construct
  REGION 1..219: note = Synthetic Construct
DIVMTQSPDSLAVSLGERATINCKSSQSLLNSRTRKNYLAWYQEKPGQPPKLLIYWASTRKSGVPDRFSGSGSGTDFTLTISSLQAEDVAVYYCKQSFILRTFGQGTKVEIKRTVAAPSVFIFPPSDEQLKSGTASVKCLLNNFYPREAKVQWKVDNALQSGNSQESVTEQDSKDSTYSLSSTLTLSKADYEKHKVYACEVTHQGLSSPVTKSFNRGEC

SEQ ID NO: 58 - protein, 14 aa, synthetic construct
  REGION 1..14: note = Synthetic Construct
WVRKAPGKGLEWVS

SEQ ID NO: 59 - protein, 112 aa, synthetic construct
  REGION 1..112: note = Synthetic Construct
EVQLLESGGGLVQPGGSLRLSCAASGFDFVNNAMIWVRKAPGKGLEWVSALSFADNTAYYATWASGRFTISRDSSKTTVYLQMNSLRAEDTAVYYCMRGDLWGPGTLVTVSS

SEQ ID NO: 60 - protein, 111 aa, synthetic construct
  REGION 1..111: note = Synthetic Construct
DIQMTQSPSTLSASVGDRVTITCQASESITRYLNWYQEKPGKAPKLLIYDASKLPSGVPSRFSGSGSGTEFTLTISSLQPDDFATYYCQSTSFRGRSYQNTFGGGTKVEIK

SEQ ID NO: 61 - protein, 15 aa, synthetic construct
  REGION 1..15: note = Synthetic Construct
WYQEKPGKAPKLLIY

SEQ ID NO: 62 - protein, 14 aa, synthetic construct
  REGION 1..14: note = Synthetic Construct
WVRKAPGQGLEWIG

SEQ ID NO: 63 - protein, 15 aa, synthetic construct
  REGION 1..15: note = Synthetic Construct
WYQQEPGQPPKLLIY

SEQ ID NO: 64 - protein, 442 aa, synthetic construct
  REGION 1..442: note = Synthetic Construct
EVQLLESGGGLVQPGGSLRLSCAASGFDFVNNAMIWVRKAPGKGLEWVSALSFADNTAYYATWASGRFTISRDSSKTTVYLQMNSLRAEDTAVYYCMRGDLWGPGTLVTVSSASTKGPSVFPLAPSSKSTSGGTAALGCLVKDYFPEPVTVSWNSGALTSGVHTFPAVLQSSGLYSLESVVTVPSSSLGTQTYICNVNHKPSNTKVDKKVEPKSCDKTHTCPPCPAPELLGGPSVFLFPPKPKDTLMISRTPEVTCVVVDVSHEDPEVKFNWYVDGVEVHNAKTKPREEQYGSTYRVVSVLTVLHQDWLNGKEYKCKVSNKALPAPIEKTISKAKGQPREPQVYTLPPSREEMTKNQVSLWCLVKGFYPSDIAVEWESNGQPENNYKTTPPVLDSDGSFFLYSKLTVDKSRWQQGNVFSCSVMHEALHNHYTQKSLSLSPGK

SEQ ID NO: 65 - protein, 218 aa, synthetic construct
  REGION 1..218: note = Synthetic Construct
DIQMTQSPSTLSASVGDRVTITCQASESITRYLNWYQEKPGKAPKLLIYDASKLPSGVPSRFSGSGSGTEFTLTISSLQPDDFATYYCQSTSFRGRSYQNTFGGGTKVEIKRTVAAPSVFIFPPSDEQLKSGTASVKCLLNNFYPREAKVQWKVDNALQSGNSQESVTEQDSKDSTYSLSSTLTLSKADYEKHKVYACEVTHQGLSSPVTKSFNRGEC

SEQ ID NO: 66 - protein, 442 aa, synthetic construct
  REGION 1..442: note = Synthetic Construct
EVQLLESGGGLVQPGGSLRLSCAASGFDFVNNAMIWVRKAPGKGLEWVSALSFADNTAYYATWASGRFTISRDSSKTTVYLQMNSLRAEDTAVYYCMRGDLWGPGTLVTVSSASTKGPSVFPLAPSSKSTSGGTAALGCLVKDYFPEPVTVSWNSGALTSGVHTFPAVLQSSGLYSLESVVTVPSSSLGTQTYICNVNHKPSNTKVDKKVEPKSCDKTHTCPPCPAPELLGGPSVFLFPPKPKDTLMISRTPEVTCVVVDVSHEDPEVKFNWYVDGVEVHNAKTKPREEQYGSTYRVVSVLTVLHQDWLNGKEYKCKVSNKALPAPIEKTISKAKGQPREPQVYTLPPSREEMTKNQVSLSCAVKGFYPSDIAVEWESNGQPENNYKTTPPVLDSDGSFFLVSKLTVDKSRWQQGNVFSCSVMHEALHNHYTQKSLSLSPGK

SEQ ID NO: 67 - protein, 449 aa, synthetic construct
  REGION 1..449: note = Synthetic Construct
EVQLVQSGAEVKKPGASVKVSCKASGFTFTSYYIHWVRKAPGQGLEWIGWIYPENDNTKYNEKFKDRVTITADTSTSTAYLELSSLRSEDTAVYYCARDGYSRYYFDYWGQGTLVTVSSASTKGPSVFPLAPSSKSTSGGTAALGCLVKDYFPEPVTVSWNSGALTSGVHTFPAVLQSSGLYSLESVVTVPSSSLGTQTYICNVNHKPSNTKVDKKVEPKSCDKTHTCPPCPAPELLGGPSVFLFPPKPKDTLMISRTPEVTCVVVDVSHEDPEVKFNWYVDGVEVHNAKTKPREEQYGSTYRVVSVLTVLHQDWLNGKEYKCKVSNKALPAPIEKTISKAKGQPREPQVYTLPPSREEMTKNQVSLWCLVKGFYPSDIAVEWESNGQPENNYKTTPPVLDSDGSFFLYSKLTVDKSRWQQGNVFSCSVMHEALHNHYTQKSLSLSPGK

SEQ ID NO: 68 - protein, 449 aa, synthetic construct
  REGION 1..449: note = Synthetic Construct
EVQLVQSGAEVKKPGASVKVSCKASGFTFTSYYIHWVREAPGQGLEWIGWIYPENDNTKYNEKFKDRVTITADTSTSTAYLELSSLRSEDTAVYYCARDGYSRYYFDYWGQGTLVTVSSASTKGPSVFPLAPSSKSTSGGTAALGCLVKDYFPEPVTVSWNSGALTSGVHTFPAVLQSSGLYSLKSVVTVPSSSLGTQTYICNVNHKPSNTKVDKKVEPKSCDKTHTCPPCPAPELLGGPSVFLFPPKPKDTLMISRTPEVTCVVVDVSHEDPEVKFNWYVDGVEVHNAKTKPREEQYGSTYRVVSVLTVLHQDWLNGKEYKCKVSNKALPAPIEKTISKAKGQPREPQVYTLPPSREEMTKNQVSLWCLVKGFYPSDIAVEWESNGQPENNYKTTPPVLDSDGSFFLYSKLTVDKSRWQQGNVFSCSVMHEALHNHYTQKSLSLSPGK

SEQ ID NO: 69 - protein, 449 aa, synthetic construct
  REGION 1..449: note = Synthetic Construct
EVQLVQSGAEVKKPGASVKVSCKASGFTFTSYYIHWVREAPGQGLEWIGWIYPENDNTKYNEKFKDRVTITADTSTSTAYLELSSLRSEDTAVYYCARDGYSRYYFDYWGQGTLVTVSSASTKGPSVFPLAPSSKSTSGGTAALGCLVKDYFPEPVTVSWNSGALTSGVHTFPAVLQSSGLYSLKSVVTVPSSSLGTQTYICNVNHKPSNTKVDKKVEPKSCDKTHTCPPCPAPELLGGPSVFLFPPKPKDTLMISRTPEVTCVVVDVSHEDPEVKFNWYVDGVEVHNAKTKPREEQYGSTYRVVSVLTVLHQDWLNGKEYKCKVSNKALPAPIEKTISKAKGQPREPQVYTLPPSREEMTKNQVSLSCAVKGFYPSDIAVEWESNGQPENNYKTTPPVLDSDGSFFLVSKLTVDKSRWQQGNVFSCSVMHEALHNHYTQKSLSLSPGK

SEQ ID NO: 70 - protein, 219 aa, synthetic construct
  REGION 1..219: note = Synthetic Construct
DIVMTQSPDSLAVSLGERATINCKSSQSLLNSRTRKNYLAWYQKKPGQPPKLLIYWASTRESGVPDRFSGSGSGTDFTLTISSLQAEDVAVYYCTQSFILRTFGQGTKVEIKRTVAAPSVFIFPPSDEQLKSGTASVECLLNNFYPREAKVQWKVDNALQSGNSQESVTEQDSKDSTYSLSSTLTLSKADYEKHKVYACEVTHQGLSSPVTKSFNRGEC

SEQ ID NO: 71-72 - skipped (2 entries)

SEQ ID NO: 73 - protein, 219 aa, synthetic construct
  REGION 1..219: note = Synthetic Construct
DIVMTQSPDSLAVSLGERATINCKSSQSLLNSRTRKNYLAWYQKKPGQPPKLLIYWASTRKSGVPDRFSGSGSGTDFTLTISSLQAEDVAVYYCKQSFILRTFGQGTKVEIKRTVAAPSVFIFPPSDEQLKSGTASVECLLNNFYPREAKVQWKVDNALQSGNSQESVTEQDSKDSTYSLSSTLTLSKADYEKHKVYACEVTHQGLSSPVTKSFNRGEC

SEQ ID NO: 74 - skipped

SEQ ID NO: 75 - protein, 133 aa, synthetic construct
  REGION 1..133: note = Synthetic Construct
MKPQFVGILLSSLLGAALGNRMRCYNCGGSPSSSCKEAVTTCGEGRPQPGLEQIKLPGNPPVTLIHQHPACVAAHHCNQVETESVGDVTYPAHRDCYLGDLCNSAVASHVAPAGILAAAATALTCLLPGLWSG

SEQ ID NO: 76 - DNA, 2449 bp, synthetic construct
  misc_feature 1..2449: note = Synthetic Construct
  source 1..2449: mol_type = other DNA
atgaaaccccagtttgttgggatcttgctcagctccctgctaggggctgccttgggtaaggaggcggccagctagcttctcacacaggccttctgccagccggctccaccgagggcccaggtccagcgcctcttttctcctgccaggaaaccgaatgcggtgctacaactgtggtggaagccccagcagttcttgcaaagaggccgtgaccacctgtggcgagggcagaccccagccaggcctggaacagatcaagctacctggaaaccgtgagtcctcagtttctccctcttccagcagcctttccctgcctccagccccatgtcaatccttctggcttccagaaccctccaggctcagtctggctctgggcagatggtgcagctgttagaggagagcagtctgtaccccttctggctcctggcacggagcccctgagaggcccacagtccttgtgcccccacttccccacctccttattctcctaaaagaatctcataggcccattagctcacaaatgaagagctctggccctgaaaggccaaagttaaaaccaaacttcaaattttcggcattagttaaggaccagggaggggtgtgtgtgtgtgtgtgtgtgtgtgtgtgtgtgtgtgtgtacatgtttttaatattttattttaacataattttggattgacagaaaagttgcagaaatactcaacttctcctaatgctaacatcttacataaccatagcacaattatcaaaatcacaaaataactgatacaatactactaactaatctacagactttatttgatttagcaagatcctacattgcatttagctctcatgtcttcttagtctcctctgatctgtgccagttctgtttttctttgtctttcatgaccctgacacatttgaagagccctgataaattattttatacctggagtttaaaaaattacttttagggccagtgcagtcactcgcacctgtaatcccagcactttaggaggccaaggtgggaggaccacttgagcccaagagttgagaccagcctgggcaacatagggagaccctgtctctacaaaaaacaaacaaacaaacaaacaaacagattaaaaaattagttgggtgtggtggcacatgcttgtagtcctagctactcagggggctgaagagggaggatcgcttgagcctgggagattgaagctacaatgagccatgatcacgccactacactccagcctggggaacaaaatgagaccctgtctcaaaaataataataataataatttttaggctaggcttggtggcacacacttgtaatcccagcactttgggaggccaaggctgaagagtcacctgaggtcaggagtttgacaccagcctgggcagcaaagtgagacccccatctctacaaaaaatgtttttaaaaaattagccaggcatagtggcacacacctgtaatctcagtttcctgagaggctgaggcaggaggattacttgagcccaggagtttgaggctatagggaggtatgattgcaccaccacactccagcctgagtgagagagcaagatcttttctctaaaattaaataaaatcatttttagattaaacaaaaattacgtgccggatgcagtggctcacgcctgtaatcccagcactttgggaggccaaggcgggtggataacctgaggtcgggagttcaagaccagcctgatcaatgtggagaaatctcgtctctactaaaaatacaaaattagccgggtgtagtggtgcccgcctgtaataccagctactcgggaacctgaggcaggagaattgcttgaacccaagaggtggaggtcgcggtgagccgagatcacaccattgcactccagctgggcaataagagtgaaactccgtctcaaaaaaaaaaaaaaaattacagatacttgaaatactaaaaattattttatagaatgtccctcgatatttatttatctgatatttgccatgatgagattgaggtcatgcattttaagcaagaatactgcagaagtgatgttgcatccttcttgctgcatcacatcaggagtttacaaggtcaatgcattaactttgatcacttggtttcagggaggtgttttttgagggggctgaaaatccctttgggctccttgaaatcacatctgctctgccccagaaggcaagtcctgaagccaggagtccaacaccccagtttcattctctctctcagccccagtgaccttgattcaccaacatccagcctgcgtcgcagcccatcattgcaatcaagtggagacagagtcggtgggagacgtgacttatccagcccacagggactgctacctgggagacctgtgcaacagcgccgtggcaagccatgtggcccctgcaggcattttggctgcagcagctaccgccctgacctgtctcttgccaggactgtggagcggatag

SEQ ID NO: 77 - protein, 133 aa, synthetic construct; identical to SEQ ID NO: 75
  REGION 1..133: note = Synthetic Construct

SEQ ID NO: 78 - protein, 10 aa, synthetic construct
  REGION 1..10: note = Synthetic Construct
RDCYLGDLCN

SEQ ID NO: 79 - skipped

SEQ ID NO: 80 - protein, 207 aa, synthetic construct
  REGION 1..207: note = Synthetic Construct
MQSGTHWRVLGLCLLSVGVWGQDGNEEMGGITQTPYKVSISGTTVILTCPQYPGSEILWQHNDKNIGGDEDDKNIGSDEDHLSLKEFSELEQSGYYVCYPRGSKPEDANFYLYLRARVCENCMEMDVMSVATIVIVDICITGGLLLLVYYWSKNRKAKAKPVTRGAGAGGRQRGQNKERPPPVPNPDYEPIRKGQRDLYSGLNQRRI

SEQ ID NO: 81 - protein, 198 aa, synthetic construct
  REGION 1..198: note = Synthetic Construct
MQSGTRWRVLGLCLLSIGVWGQDGNEEMGSITQTPYQVSISGTTVILTCSQHLGSEAQWQHNGKNKEDSGDRLFLPEFSEMEQSGYYVCYPRGSNPEDASHHLYLKARVCENCMEMDVMAVATIVIVDICITLGLLLLVYYWSKNRKAKAKPVTRGAGAGGRQRGQNKERPPPVPNPDYEPIRKGQQDLYSGLNQRRI

SEQ ID NO: 82 - protein, 182 aa, synthetic construct
  REGION 1..182: note = Synthetic Construct
MEQGKGLAVLILAIILLQGTLAQSIKGNHLVKVYDYQEDGSVLLTCDAEAKNITWFKDGKMIGFLTEDKKKWNLGSNAKDPRGMYQCKGSQNKSKPLQVYYRMCQNCIELNAATISGFLFAEIVSIFVLAVGVYFIAGQDGVRQSRASDKQTLLPNDQLYQPLKDREDDQYSHLQGNQLRRN

SEQ ID NO: 83 - protein, 181 aa, synthetic construct
  REGION 1..181: note = Synthetic Construct
MVQGKGLTGFILAIILLQGSLAQSFEENRKLNVYNQEDGSVLLTCHVKNTNITWFKEGKMIDILTAHKNKWNLGSNTKDPRGVYQCKGSKDKSKTLQVYYRMCQNCIELNAATILGFVFAEIISIFFLAVGVYFIAGQDGVRQSRASDKQTLLPNDQLYQPLKDREDDQYSHLQGNQLRMN

SEQ ID NO: 84 - protein, 26 aa, synthetic construct
  REGION 1..26: note = Synthetic Construct
MQSGTHWRVLGLCLLSVGVWGQDGNE

SEQ ID NO: 85 - protein, 27 aa, synthetic construct
  REGION 1..27: note = Synthetic Construct
MQSGTHWRVLGLCLLSVGVWGQDGNEE

SEQ ID NO: 86 - protein, 16 aa, synthetic construct
  REGION 1..16: note = Synthetic Construct
QDGNEEMGGITQTPYK

SEQ ID NO: 87 - protein, 12 aa, synthetic construct
  REGION 1..12: note = Synthetic Construct
HRDCYLGDLCNS

SEQ ID NO: 88 - protein, 91 aa, synthetic construct
  REGION 1..91: note = Synthetic Construct
NRMRCYNCGGSPSSSCKEAVTTCGEGRPQPGLEQIKLPGNPPVTLIHQHPACVAAHHCNQVETESVGDVTYPAHRDCYLGDLCNSAGNSVT

SEQ ID NO: 89 - protein, 119 aa, synthetic construct
  REGION 1..119: note = Synthetic Construct
EVQLVQSGAEVKKPGASVKVSCKASGFTFTSYYIHWVREAPGQGLEWIGWIYPENDNTKYNEKFKDRVTITADTSTSTAYLELSSLRSEDTAVYYCARDGYSRYYFDYWGQGTLVTVSS

SEQ ID NO: 90 - protein, 112 aa, synthetic construct
  REGION 1..112: note = Synthetic Construct
DIVMTQSPDSLAVSLGERATINCKSSQSLLNSRTRKNYLAWYQKKPGQPPKLLIYWASTRESGVPDRFSGSGSGTDFTLTISSLQAEDVAVYYCTQSFILRTFGQGTKVEIK

SEQ ID NO: 91 - skipped

SEQ ID NO: 92 - protein, 112 aa, synthetic construct
  REGION 1..112: note = Synthetic Construct
DIVMTQSPDSLAVSLGERATINCKSSQSLLNSRTRKNYLAWYQKKPGQPPKLLIYWASTRKSGVPDRFSGSGSGTDFTLTISSLQAEDVAVYYCKQSFILRTFGQGTKVEIK

SEQ ID NO: 93 - protein, 112 aa, synthetic construct
  REGION 1..112: note = Synthetic Construct
DIVMTQSPDSLAVSLGERATINCKSSQSLLNSRTRKNYLAWYQQKPGQSPKLLIYWTSTRKSGVPDRFSGSGSGTDFTLTISSLQAEDVAVYYCKQSFILRTFGQGTKVEIK

SEQ ID NO: 94 - protein, 112 aa, synthetic construct
  REGION 1..112: note = Synthetic Construct
DIVMTQSPDSLAVSLGERATINCKSSQSLLNSRTRKNYLAWYQQKPGQPPKLLIYWASTRKSGVPDRFSGSGSGTDFTLTISSLQAEDVAVYYCKQSFILRTFGQGTKVEIK

SEQ ID NO: 95 - protein, 222 aa, synthetic construct
  REGION 1..222: note = Synthetic Construct
EVQLVQSGAEVKKPGASVKVSCKASGYTFTTYVMHWVRQAPGQGLEWMGYINPYNDGTKYNEKFKGRVTMTRDTSISTAYMELSRLRSDDTAVYYCGRRNFDYWGQGTLVTVSSASTKGPSVFPLAPSSKSTSGGTAALGCLVKDYFPEPVTVSWNSGALTSGVHTFPAVLQSSGLYSLSSVVTVPSSSLGTQTYICNVNHKPSNTKVDKKVEPKSCDKTHT

SEQ ID NO: 96 - protein, 216 aa, synthetic construct
  REGION 1..216: note = Synthetic Construct
EVQLLESGGGLVQPGGSLRLSCAASGFDFVNNAMIWVRQAPGKGLEWVSALSFADNTAYYATWASGRFTISRDSSKTTVYLQMNSLRAEDTAVYYCMRGDLWGPGTLVTVSSASTKGPSVFPLAPSSKSTSGGTAALGCLVKDYFPEPVTVSWNSGALTSGVHTFPAVLQSSGLYSLSSVVTVPSSSLGTQTYICNVNHKPSNTKVDKKVEPKSCD

SEQ ID NO: 97 - protein, 218 aa, synthetic construct
  REGION 1..218: note = Synthetic Construct
DIQMTQSPSTLSASVGDRVTITCQASESITRYLNWYQQKPGKAPKLLIYDASKLPSGVPSRFSGSGSGTEFTLTISSLQPDDFATYYCQSTSFRGRSYQNTFGGGTKVEIKRTVAAPSVFIFPPSDEQLKSGTASVVCLLNNFYPREAKVQWKVDNALQSGNSQESVTEQDSKDSTYSLSSTLTLSKADYEKHKVYACEVTHQGLSSPVTKSFNRGEC

SEQ ID NO: 98 - protein, 119 aa, synthetic construct
  REGION 1..119: note = Synthetic Construct
EVQLVQSGAEVKKPGASVKVSCKASGYTFTNYYIHWVRQAPGQGLEWIGWIYPGDGNTKYNEKFKGRATLTADTSTSTAYLELSSLRSEDTAVYYCARDSYSNYYFDYWGQGTLVTVSS

SEQ ID NO: 99 - protein, 13 aa, synthetic construct
  REGION 1..13: note = Synthetic Construct
QSTSFRGRSYNNT

SEQ ID NO: 100 - protein, 13 aa, synthetic construct
  REGION 1..13: note = Synthetic Construct
QSTSFRGRSYQNV

SEQ ID NO: 101 - protein, 13 aa, synthetic construct
  REGION 1..13: note = Synthetic Construct
QSTSFRGRSYSNT

SEQ ID NO: 102 - protein, 13 aa, synthetic construct
  REGION 1..13: note = Synthetic Construct
QSTSFRGRSYSNA

SEQ ID NO: 103 - protein, 13 aa, synthetic construct
  REGION 1..13: note = Synthetic Construct
QSTSFRGRSYANT

SEQ ID NO: 104 - protein, 13 aa, synthetic construct
  REGION 1..13: note = Synthetic Construct
QSTSFRGRSYNNA

SEQ ID NO: 105 - protein, 13 aa, synthetic construct
  REGION 1..13: note = Synthetic Construct
QSTSFRGRSYNNV

SEQ ID NO: 106 - protein, 13 aa, synthetic construct
  REGION 1..13: note = Synthetic Construct
QSTSFRGRSYGNT

SEQ ID NO: 107 - protein, 13 aa, synthetic construct
  REGION 1..13: note = Synthetic Construct
QSTSFRGRSYSNV

SEQ ID NO: 108 - protein, 112 aa, synthetic construct
  REGION 1..112: note = Synthetic Construct
DIVMTQSPDSLAVSLGERATINCKSSQSLLNSRTRKNYLAWYQKKPGQSPKLLIYWTSTRKSGVPDRFSGSGSGTDFTLTISSLQAEDVAVYYCKQSFILRTFGQGTKVEIK

SEQ ID NO: 109 - protein, 119 aa, synthetic construct
  REGION 1..119: note = Synthetic Construct
EVQLVQSGAEVKKPGASVKVSCKASGYTFTNYYIHWVRKAPGQGLEWIGWIYPGDGNTKYNEKFKGRATLTADTSTSTAYLELSSLRSEDTAVYYCARDSYSNYYFDYWGQGTLVTVSS

SEQ ID NO: 110 - protein, 7 aa, synthetic construct
  REGION 1..7: note = Synthetic Construct
WASTRIS

SEQ ID NO: 111 - protein, 5 aa, synthetic construct
  REGION 1..5: note = Synthetic Construct
NNAMS

SEQ ID NO: 112 - protein, 17 aa, synthetic construct
  REGION 1..17: note = Synthetic Construct
SLSFADNTAYYATWASG

SEQ ID NO: 113 - protein, 17 aa, synthetic construct
  REGION 1..17: note = Synthetic Construct
ILSFADNTAYYATWASG

SEQ ID NO: 114 - protein, 442 aa, synthetic construct
  REGION 1..442: note = Synthetic Construct
EVQLLESGGGLVQPGGSLRLSCAASGFDFVNNAMIWVRQAPGKGLEWVSALSFADNTAYYATWASGRFTISRDSSKTTVYLQMNSLRAEDTAVYYCMRGDLWGPGTLVTVSSASTKGPSVFPLAPSSKSTSGGTAALGCLVKDYFPEPVTVSWNSGALTSGVHTFPAVLQSSGLYSLSSVVTVPSSSLGTQTYICNVNHKPSNTKVDKKVEPKSCDKTHTCPPCPAPELLGGPSVFLFPPKPKDTLMISRTPEVTCVVVDVSHEDPEVKFNWYVDGVEVHNAKTKPREEQYGSTYRVVSVLTVLHQDWLNGKEYKCKVSNKALPAPIEKTISKAKGQPREPQVYTLPPSREEMTKNQVSLWCLVKGFYPSDIAVEWESNGQPENNYKTTPPVLDSDGSFFLYSKLTVDKSRWQQGNVFSCSVMHEALHNHYTQKSLSLSPGK

SEQ ID NO: 115 - protein, 218 aa, synthetic construct; identical to SEQ ID NO: 97
  REGION 1..218: note = Synthetic Construct

SEQ ID NO: 116 - protein, 7 aa, synthetic construct
  REGION 1..7: note = Synthetic Construct
GRSYNNT

SEQ ID NO: 117 - protein, 111 aa, synthetic construct
  REGION 1..111: note = Synthetic Construct
DIQMTQSPSSLSASVGDRVTITCQASESITRYLNWYQQKPGKPPKLLIYDASKLPSGVPSRFSGSGSGTDFTLTISSLQPEDFATYYCQSTSFRGRSYNNTFGGGTKVEIK

SEQ ID NO: 118 - protein, 111 aa, synthetic construct
  REGION 1..111: note = Synthetic Construct
DIQMTQSPSTLSASVGDRVTITCQASESITRYLNWYQQKPGKPPKLLIYDASKLPSGVPSRFSGSGSGTEFTLTISSLQPDDFATYYCQSTSFRGRSYNNTFGGGTKVEIK

SEQ ID NO: 119 - protein, 111 aa, synthetic construct
  REGION 1..111: note = Synthetic Construct
DIVMTQSPDSLAVSLGERATINCQASESITRYLNWYQQKPGQPPKLLIYDASKLPSGVPDRFSGSGSGTDFTLTISSLQAEDVAVYYCQSTSFRGRSYNNTFGGGTKVEIK

SEQ ID NO: 120 - protein, 112 aa, synthetic construct
  REGION 1..112: note = Synthetic Construct
EQQLLESGGGLVQPGGSLRLSCAASGFDFVNNAMSWVRQAPGKGLEWIAALSFADNTAYYATWASGRFTISKDSSKTTVYLQMNSLRAEDTAVYFCMRGDLWGPGTLVTVSS

SEQ ID NO: 121 - protein, 112 aa, synthetic construct
  REGION 1..112: note = Synthetic Construct
EQQLVESGGGVVQPGRSLRLSCAASGFDFVNNAMSWVRQAPGKGLEWIAALSFADNTAYYATWASGRFTISKDSSKNTVYLQMNSLRAEDTAVYFCMRGDLWGPGTLVTVSS

SEQ ID NO: 122 - protein, 111 aa, synthetic construct
  REGION 1..111: note = Synthetic Construct
DIQMTQSPSTLSASVGDRVTITCQASESITRYLNWYQQKPGKPPKLLIYDASKLPSGVPSRFSGSGSGTEFTLTISSLQPDDFATYYCQSTSFRGRSYQNTFGGGTKVEIK

SEQ ID NO: 123 - protein, 112 aa, synthetic construct
  REGION 1..112: note = Synthetic Construct
EQQLVESGGGVVQPGRSLRLSCAASGFDFVNNAMIWVRQAPGKGLEWIAALSFADNTAYYATWASGRFTISKDSSKNTVYLQMNSLRAEDTAVYFCMRGDLWGPGTLVTVSS

SEQ ID NO: 124 - protein, 107 aa, synthetic construct
  REGION 1..107: note = Synthetic Construct
DIQMTQSPSTLSASVGDRVTITCRASQSISSWLAWYQQKPGKAPKLLIYDASSLESGVPSRFSGSGSGTEFTLTISSLQPDDFATYYCQQYNSYSLTFGGGTKVEIK

SEQ ID NO: 125 - protein, 112 aa, synthetic construct
  REGION 1..112: note = Synthetic Construct
EVQLLESGGGLVQPGGSLRLSCAASGFTFSSYAMSWVRQAPGKGLEWVSAISGSGGSTYYADSVKGRFTISRDNSKNTLYLQMNSLRAEDTAVYYCAKFDLWGRGTLVTVSS

SEQ ID NO: 126 - protein, 112 aa, synthetic construct
  REGION 1..112: note = Synthetic Construct
DIVMTQSPDSLAVSLGERATINCKSSQSLLNSRTRKNYLAWYQEKPGQSPKLLIYWTSTRKSGVPDRFSGSGSGTDFTLTISSLQAEDVAVYYCKQSFILRTFGQGTKVEIK

SEQ ID NO: 127 - protein, 119 aa, synthetic construct
  REGION 1..119: note = Synthetic Construct
EVQLVQSGAEVKKPGASVKVSCKASGYTFTNYYIHWVREAPGQGLEWIGWIYPGDGNTKYNEKFKGRATLTADTSTSTAYLELSSLRSEDTAVYYCARDSYSNYYFDYWGQGTLVTVSS

SEQ ID NO: 128 - protein, 112 aa, synthetic construct
  REGION 1..112: note = Synthetic Construct
DIVMTQSPDSLAVSLGERATINCKSSQSLLNSRTRKNYLAWYQQKPGQPPKLLIYWTSTRKSGVPDRFSGSGSGTDFTLTISSLQAEDVAVYYCKQSFILRTFGQGTKVEIK

SEQ ID NO: 129 - protein, 112 aa, synthetic construct
  REGION 1..112: note = Synthetic Construct
DIVMTQSPDSLAVSLGERATINCKSSQSLLNSRTRKNYLAWYQQKPGQSPKLLIYWASTREKGVPDRFSGSGSGTDFTLTISSLQAEDVAVYYCKQSFILRTFGQGTKVEIK

SEQ ID NO: 130 - protein, 111 aa, synthetic construct
  REGION 1..111: note = Synthetic Construct
DIVMTQTPSSVSAAVGGTVTINCQASESITRYLNWYQQKPGQPPKLLIYDASKLPSGVPSRFKGSGSGTQFTLTTSDLECADAATYYCQSTSFRGRSYNNTFGGGTEVVVK

SEQ ID NO: 131 - protein, 111 aa, synthetic construct
  REGION 1..111: note = Synthetic Construct
QQQLEESGGDLVKPGASLTLTCTASGFDFVNNAMCWVRQAPGKGLEWIACLSFADNTAYYATWASGRFTISKISSTTVTLRMTSLTGADTATYFCMRGDLWGPGTLVTVSS

SEQ ID NO: 132 - protein, 111 aa, synthetic construct
  REGION 1..111: note = Synthetic Construct
EAVLTQSPGTLSLSPGERATLSCQSSESVWHNNWLAWFQQKPGQRPRLLIYGASTLASGVPDRFSGSGSGTDFTLTISRLEPEDFAVYYCAGGYSSSDAHVFGGGTKVEIK

SEQ ID NO: 133 - protein, 111 aa, synthetic construct
  REGION 1..111: note = Synthetic Construct
DAQLTQSPSTLSASVGDRVTITCQSSESVWHNNWLAWFQQKPGKRPKLLIYGASTLASGVPSRFSGSGSGTEFTLTISSLQPDDFATYYCAGGYSSSDAHVFGGGTKVEIK

SEQ ID NO: 134 - protein, 111 aa, synthetic construct
  REGION 1..111: note = Synthetic Construct
DAVLTQSPDSLAVSLGERATINCQSSESVWHNNWLAWFQQKPGQRPKLLIYGASTLASGVPDRFSGSGSGTDFTLTISSLQAEDVAVYYCAGGYSSSDAHVFGGGTKVEIK

SEQ ID NO: 135 - protein, 118 aa, synthetic construct
  REGION 1..118: note = Synthetic Construct
EQQLVESGGGLIQPGGSLRLSCAVSGLSLSTNSINWVRQAPGKGLEWIGYIYHGDGIADYASWAKGRFTISKDSSKNTVYLQMNSLRAEDTAVYFCASGAGYSLFTLWGPGTLVTVSS

SEQ ID NO: 136 - protein, 118 aa, synthetic construct
  REGION 1..118: note = Synthetic Construct
EQQLQESGPGLVKPPGTLSLTCAVSGLSLSTNSINWVRQPPGKGLEWIGYIYHGDGIADYASWAKGRFTISKDSSKTQVSLKLSSVTAADTAVYFCASGAGYSLFTLWGPGTLVTVSS

SEQ ID NO: 137 - protein, 118 aa, synthetic construct
  REGION 1..118: note = Synthetic Construct
EQQLVESGGGLVQPGGSLRLSCAVSGLSLSTNSINWVRQAPGKGLEWIGYIYHGDGIADYASWAKGRFTISKDSAKNSVYLQMNSLRAEDTAVYFCASGAGYSLFTLWGPGTLVTVSS

SEQ ID NO: 138 - protein, 111 aa, synthetic construct
  REGION 1..111: note = Synthetic Construct
AAVLTQTPSPVSAAVGGTITINCQSSESVWHNNWLAWFQQKPGQRPRLLIYGASTLASGVPSRFSGTGSGTQFTLTISDVQCDDAATYYCAGGYSSSDAHVFGRGTAVVVK

SEQ ID NO: 139 - protein, 111 aa, synthetic construct
  REGION 1..111: note = Synthetic Construct
DAQMTQSPSTLSASVGDRVTITCQSSESVWHNNWLAWFQQKPGKRPKLLIYGASTLASGVPSRFSGSGSGTEFTLTISSLQPDDFATYYCAGGYSSSDAHVFGGGTKVEIK

SEQ ID NO: 140 - protein, 111 aa, synthetic construct
  REGION 1..111: note = Synthetic Construct
EAVLTQSPGTLSLSPGERATLSCQSSESVWHNNWLAWFQQKPGQAPRLLIYGASTLASGVPDRFSGSGSGTDFTLTISRLEPEDFAVYYCAGGYSSSDAHVFGGGTKVEIK

SEQ ID NO: 141 - protein, 116 aa, synthetic construct
  REGION 1..116: note = Synthetic Construct
QSLEESGGGLVKPGGTLTLTCTVSGLSLSTNSINWVRQAPGKGLEWIGYIYHGDGIADYASWAKGRFTISKTSSTTVTLRMTSLTVADTATYFCASGAGYSLFTLWGPGTLVTVSS

SEQ ID NO: 142 - protein, 118 aa, synthetic construct
  REGION 1..118: note = Synthetic Construct
EVQLVESGGGLVQPGGSLRLSCAASGLSLSTNSINWVRQAPGKGLEWVSYIYHGDGIADYASWAKGRFTISRDNAKNSLYLQMNSLRAEDTAVYYCASGAGYSLFTLWGRGTLVTVSS

SEQ ID NO: 143 - protein, 118 aa, synthetic construct
  REGION 1..118: note = Synthetic Construct
EVQLVESGGGLIQPGGSLRLSCAASGLSLSTNSINWVRQAPGKGLEWVSYIYHGDGIADYASWAKGRFTISRDNSKNTLYLQMNSLRAEDTAVYYCASGAGYSLFTLWGRGTLVTVSS

SEQ ID NO: 144 - protein, 108 aa, synthetic construct
  REGION 1..108: note = Synthetic Construct
EIVLTQSPGTLSLSPGERATLSCRASQSVSSSYLAWYQQKPGQAPRLLIYGASSRATGIPDRFSGSGSGTDFTLTISRLEPEDFAVYYCQQYGSSPLTFGGGTKVEIK

SEQ ID NO: 145 - protein, 111 aa, synthetic construct
  REGION 1..111: note = Synthetic Construct
EVQLVESGGGLIQPGGSLRLSCAASGFTVSSNYMSWVRQAPGKGLEWVSVIYSGGSTYYADSVKGRFTISRDNSKNTLYLQMNSLRAEDTAVYYCARFDLWGRGTLVTVSS

SEQ ID NO: 146 - protein, 112 aa, synthetic construct
  REGION 1..112: note = Synthetic Construct
EVQLVESGGGLVQPGGSLRLSCAASGFTFSSYSMNWVRQAPGKGLEWVSYISSSSSTIYYADSVKGRFTISRDNAKNSLYLQMNSLRAEDTAVYYCARFDLWGRGTLVTVSS

SEQ ID NO: 147 - protein, 220 aa, synthetic construct
  REGION 1..220: note = Synthetic Construct
DIVMTQSPDSLAVSLGERATINCKSSQSLLLSGNQENYLAWHQQKPGQPPKTLITWASTRISGVPDRFSGSGSGTDFTLTISSLQAEDVAVYYCQQSYSAPYTFGGGTKVEIKRTVAAPSVFIFPPSDEQLKSGTASVVCLLNNFYPREAKVQWKVDNALQSGNSQESVTEQDSKDSTYSLSSTLTLSKADYEKHKVYACEVTHQGLSSPVTKSFNRGEC